European Patent Application EP 4 644 549 A1, published November 5, 2025. Title: 抗菌ペプチドおよびその製造方法. Applicant: 住友化学株式会社. The sequence listing filed with the application follows.

SEQUENCE LISTING (32 sequences)

SEQ ID NO: 1 - protein, 27 aa, Lactiplantibacillus plantarum
MSKKQWYRLGERVGRVAVFIGGGLLFK

SEQ ID NO: 2 - protein, 28 aa, Lactiplantibacillus plantarum
KTKTISLMSGLQVPHAFTKLLKALGGHH

SEQ ID NO: 3 - protein, 31 aa, Lactiplantibacillus plantarum
WLQYLIPVVVSGLNHTDQIMRGWKKGYHRHH

SEQ ID NO: 4 - protein, 40 aa, Lactiplantibacillus plantarum
SSSLLNTAWRKFGQIAGTVTSAGLDAGWIRAHKYGHGRSH

SEQ ID NO: 5 - protein, 31 aa, Lactiplantibacillus plantarum
  VARIANT 23: note = A or V
SHAYNAAAIRRNNKSMKGAASFXKKFFPAFF

SEQ ID NO: 6 - protein, 22 aa, Lactiplantibacillus plantarum
FKSWSLCTFGCGHTGSFNSFCC

SEQ ID NO: 7 - DNA, 84 bp, Lactiplantibacillus plantarum
  source 1..84: mol_type = genomic DNA
  CDS 1..84: protein_id = 1; translation = MSKKQWYRLGERVGRVAVFIGGGLLFK
atgagtaaaaagcaatggtatcgtttaggagaacgtgtcggtcgtgtagcagtttttatcggtggaggattactttttaaataa

SEQ ID NO: 8 - DNA, 87 bp, Lactiplantibacillus plantarum
  source 1..87: mol_type = genomic DNA
  CDS 1..87: protein_id = 2; translation = KTKTISLMSGLQVPHAFTKLLKALGGHH
aaaacaaagactataagcttgatgtcggggttgcaagtcccccatgcttttacaaaattattgaaagcacttggaggccatcattag

SEQ ID NO: 9 - DNA, 96 bp, Lactiplantibacillus plantarum
  source 1..96: mol_type = genomic DNA
  CDS 1..96: protein_id = 3; translation = WLQYLIPVVVSGLNHTDQIMRGWKKGYHRHH
tggctacaatacctgatccctgttgtggttagcggcctcaatcatacagaccaaattatgcgtggttggaaaaaaggataccatcgtcatcattag

SEQ ID NO: 10 - DNA, 123 bp, Lactiplantibacillus plantarum
  source 1..123: mol_type = genomic DNA
  CDS 1..123: protein_id = 4; translation = SSSLLNTAWRKFGQIAGTVTSAGLDAGWIRAHKYGHGRSH
tctagcagtcttttaaatactgcatggcggaaatttggtcaaatagctggtaccgttacttctgcaggattggatgcaggttggatcagggctcataagtatggacatggtaggagtcactag

SEQ ID NO: 11 - DNA, 96 bp, Lactiplantibacillus plantarum
  source 1..96: mol_type = genomic DNA
  CDS 1..96: protein_id = 5; translation = SHAYNAAAIRRNNKSMKGAASFXKKFFPAFF
tctcacgcatataacgctgctgctattcgtagaaataacaaatctatgaaaggcgccgcaagttttgytaagaaattctttcctgcctttttttga

SEQ ID NO: 12 - DNA, 69 bp, Lactiplantibacillus plantarum
  source 1..69: mol_type = genomic DNA
  CDS 1..69: protein_id = 6; translation = FKSWSLCTFGCGHTGSFNSFCC
tttaagagttggtcactttgcacctttggctgtggtcacacaggcagctttaatagtttctgttgctaa

SEQ ID NO: 13 - protein, 36 aa, Lactiplantibacillus plantarum
SNNKFWTWAGYTYENWRISSRRAFNLRQRKNTMTHH

SEQ ID NO: 14 - protein, 37 aa, Lactiplantibacillus plantarum
IWQWIVGGLGFLAGDAWSHSDQISSGIKKRKKKGYGY

SEQ ID NO: 15 - DNA, 111 bp, Lactiplantibacillus plantarum
  source 1..111: mol_type = genomic DNA
  CDS 1..111: protein_id = 13; translation = SNNKFWTWAGYTYENWRISSRRAFNLRQRKNTMTHH
agtaataataagttttggacttgggctggttacacatatgagaattggcgtatttcatcaaggcgagcgtttaatctacgtcagcgcaaaaacactatgactcatcattag

SEQ ID NO: 16 - DNA, 114 bp, Lactiplantibacillus plantarum
  source 1..114: mol_type = genomic DNA
  CDS 1..114: protein_id = 14; translation = IWQWIVGGLGFLAGDAWSHSDQISSGIKKRKKKGYGY
atttggcaatggattgtgggcggtttaggctttcttgctggtgatgcatggtcccattcagatcaaatctcaagtggaattaagaaacgcaagaaaaaaggttatggctactag

SEQ ID NO: 17 - DNA, 138 bp, Lactiplantibacillus plantarum
  source 1..138: mol_type = genomic DNA
  CDS 1..138: protein_id = 25; translation = MNKYVELDLEQLQQISGGMSKKQWYRLGERVGRVAVFIGGGLLFK
atgaacaaatatgtcgaacttgatttagaacaattgcaacaaatctcaggcggtatgagtaaaaagcaatggtatcgtttaggagaacgtgtcggtcgtgtagcagtttttatcggtggaggattactttttaaataa

SEQ ID NO: 18 - DNA, 150 bp, Lactiplantibacillus plantarum
  source 1..150: mol_type = genomic DNA
  CDS 1..150: protein_id = 26; translation = MKNINKYTELNDQKLQSLIGGKTKTISLMSGLQVPHAFTKLLKALGGHH
atgaaaaacattaataagtacactgaactaaatgatcagaagttgcaatctttaattggcggaaaaacaaagactataagcttgatgtcggggttgcaagtcccccatgcttttacaaaattattgaaagcacttggaggccatcattag

SEQ ID NO: 19 - DNA, 168 bp, Lactiplantibacillus plantarum
  source 1..168: mol_type = genomic DNA
  CDS 1..168: protein_id = 27; translation = MKNLSSLNQFKTIDAKQQANISGGWLQYLIPVVVSGLNHTDQIMRGWKKGYHRHH
atgaaaaatctaagttctttaaatcaatttaagacgattgatgctaagcaacaggctaacatctcaggtggatggctacaatacctgatccctgttgtggttagcggcctcaatcatacagaccaaattatgcgtggttggaaaaaaggataccatcgtcatcattag

SEQ ID NO: 20 - DNA, 177 bp, Lactiplantibacillus plantarum
  source 1..177: mol_type = genomic DNA
  CDS 1..177: protein_id = 28; translation = MQNFSSIKTEELQAIVGGSSSLLNTAWRKFGQIAGTVTSAGLDAGWIRAHKYGHGRSH
atgcaaaattttagtagtattaaaactgaagaactacaggcaatagttggggggtctagcagtcttttaaatactgcatggcggaaatttggtcaaatagctggtaccgttacttctgcaggattggatgcaggttggatcagggctcataagtatggacatggtaggagtcactag

SEQ ID NO: 21 - DNA, 153 bp, Lactiplantibacillus plantarum
  source 1..153: mol_type = genomic DNA
  CDS 1..153: protein_id = 29; translation = MKSNYKNLSDNSLKRILGGSHAYNAAAIRRNNKSMKGAASFXKKFFPAFF
atgaaaagtaactataaaaatttatcagataatagtcttaaaaggattttaggtggatctcacgcatataacgctgctgctattcgtagaaataacaaatctatgaaaggcgccgcaagttttgytaagaaattctttcctgcctttttttga

SEQ ID NO: 22 - DNA, 189 bp, Lactiplantibacillus plantarum
  source 1..189: mol_type = genomic DNA
  CDS 1..189: protein_id = 30; translation = MLENNETNTQTLDLNDALFDLDVTENEASVVKDEDDPDSRFKSWSLCTFGCGHTGSFNSFCC
atgttagaaaataatgagacaaatacgcagactttggacttaaatgatgctttgtttgatttagatgttaccgaaaatgaggcttcagtcgttaaagatgaggatgacccagattcacgctttaagagttggtcactttgcacctttggctgtggtcacacaggcagctttaatagtttctgttgctaa

SEQ ID NO: 23 - DNA, 174 bp, Lactiplantibacillus plantarum
  source 1..174: mol_type = genomic DNA
  CDS 1..174: protein_id = 31; translation = MKNINNFQALQKNELSKVKGGSNNKFWTWAGYTYENWRISSRRAFNLRQRKNTMTHH
atgaaaaatattaataattttcaggcattgcaaaaaaatgagctttctaaagttaaaggtggtagtaataataagttttggacttgggctggttacacatatgagaattggcgtatttcatcaaggcgagcgtttaatctacgtcagcgcaaaaacactatgactcatcattag

SEQ ID NO: 24 - DNA, 180 bp, Lactiplantibacillus plantarum
  source 1..180: mol_type = genomic DNA
  CDS 1..180: protein_id = 32; translation = MRKSISNFKALNEKELGAVNGGIWQWIVGGLGFLAGDAWSHSDQISSGIKKRKKKGYGY
atgagaaaaagcatcagtaattttaaagcattaaatgaaaaagaacttggcgctgttaacggtgggatttggcaatggattgtgggcggtttaggctttcttgctggtgatgcatggtcccattcagatcaaatctcaagtggaattaagaaacgcaagaaaaaaggttatggctactag

SEQ ID NO: 25 - protein, 45 aa, Lactiplantibacillus plantarum
MNKYVELDLEQLQQISGGMSKKQWYRLGERVGRVAVFIGGGLLFK

SEQ ID NO: 26 - protein, 49 aa, Lactiplantibacillus plantarum
MKNINKYTELNDQKLQSLIGGKTKTISLMSGLQVPHAFTKLLKALGGHH

SEQ ID NO: 27 - protein, 55 aa, Lactiplantibacillus plantarum
MKNLSSLNQFKTIDAKQQANISGGWLQYLIPVVVSGLNHTDQIMRGWKKGYHRHH

SEQ ID NO: 28 - protein, 58 aa, Lactiplantibacillus plantarum
MQNFSSIKTEELQAIVGGSSSLLNTAWRKFGQIAGTVTSAGLDAGWIRAHKYGHGRSH

SEQ ID NO: 29 - protein, 50 aa, Lactiplantibacillus plantarum
  VARIANT 42: note = A or V
MKSNYKNLSDNSLKRILGGSHAYNAAAIRRNNKSMKGAASFXKKFFPAFF

SEQ ID NO: 30 - protein, 62 aa, Lactiplantibacillus plantarum
MLENNETNTQTLDLNDALFDLDVTENEASVVKDEDDPDSRFKSWSLCTFGCGHTGSFNSFCC

SEQ ID NO: 31 - protein, 57 aa, Lactiplantibacillus plantarum
MKNINNFQALQKNELSKVKGGSNNKFWTWAGYTYENWRISSRRAFNLRQRKNTMTHH

SEQ ID NO: 32 - protein, 59 aa, Lactiplantibacillus plantarum
MRKSISNFKALNEKELGAVNGGIWQWIVGGLGFLAGDAWSHSDQISSGIKKRKKKGYGY